European Patent Application EP 4 775 987 A2, published July 15, 2026. Title: METHODS AND COMPOSITIONS FOR DIAGNOSIS AND TREATMENT OF DISORDERS IN PATIENTS WITH ELEVATED LEVELS OF CXCL9 AND OTHER BIOMARKERS. Applicant: SWEDISH ORPHAN BIOVITRUM AG. Application EP. The sequence listing filed with the application follows.

SEQUENCE LISTING (105 sequences)

SEQ ID NO: 1 - protein, 5 aa, synthetic construct
SYAMS

SEQ ID NO: 2 - protein, 17 aa, synthetic construct
AISGSGGSTYYADSVKG

SEQ ID NO: 3 - protein, 14 aa, synthetic construct
DGSSGWYVPHWFDP

SEQ ID NO: 4 - protein, 13 aa, synthetic construct
TRSSGSIASNYVQ

SEQ ID NO: 5 - protein, 7 aa, synthetic construct
EDNQRPS

SEQ ID NO: 6 - protein, 10 aa, synthetic construct
QSYDGSNRWM

SEQ ID NO: 7 - protein, 13 aa, synthetic construct
TRSSGSIVSNYVQ

SEQ ID NO: 8 - protein, 7 aa, synthetic construct
EDNRRPS

SEQ ID NO: 9 - protein, 14 aa, synthetic construct
DHSSGWYVISGMDV

SEQ ID NO: 10 - protein, 9 aa, synthetic construct
QSNDSDNVV

SEQ ID NO: 11 - protein, 13 aa, synthetic construct
DLTVGGPWYYFDY

SEQ ID NO: 12 - protein, 7 aa, synthetic construct
DDDQRPS

SEQ ID NO: 13 - protein, 9 aa, synthetic construct
QSYDSSNVV

SEQ ID NO: 14 - protein, 11 aa, synthetic construct
DGWNALGWLES

SEQ ID NO: 15 - protein, 13 aa, synthetic construct
TRSGGSIGSYYVQ

SEQ ID NO: 16 - protein, 7 aa, synthetic construct
DDKKRPS

SEQ ID NO: 17 - protein, 10 aa, synthetic construct
QSYDSNNLVV

SEQ ID NO: 18 - protein, 13 aa, synthetic construct
TRSSGTIASNYVQ

SEQ ID NO: 19 - protein, 10 aa, synthetic construct
QSYDNSNHWV

SEQ ID NO: 20 - protein, 5 aa, synthetic construct
SNAMS

SEQ ID NO: 21 - protein, 17 aa, synthetic construct
TLTGSGGTAYYADSVEG

SEQ ID NO: 22 - protein, 11 aa, synthetic construct
GTELVGGGLDN

SEQ ID NO: 23 - protein, 13 aa, synthetic construct
TGSGGSIATNYVQ

SEQ ID NO: 24 - protein, 11 aa, synthetic construct
QSYDSDNHHVV

SEQ ID NO: 25 - protein, 13 aa, synthetic construct
TGSSGSIASNYVQ

SEQ ID NO: 26 - protein, 11 aa, synthetic construct
QSYDSSNQEVV

SEQ ID NO: 27 - protein, 10 aa, synthetic construct
QSYDSNNFWV

SEQ ID NO: 28 - protein, 11 aa, synthetic construct
RSFDSGGSFEY

SEQ ID NO: 29 - protein, 7 aa, synthetic construct
EDDRRPS

SEQ ID NO: 30 - protein, 10 aa, synthetic construct
QSYDDTTPWV

SEQ ID NO: 31 - protein, 11 aa, synthetic construct
VGSWYLEDFDI

SEQ ID NO: 32 - protein, 13 aa, synthetic construct
TRSSGSIASNYVH

SEQ ID NO: 33 - protein, 12 aa, synthetic construct
QSSDTTYHGGVV

SEQ ID NO: 34 - protein, 13 aa, synthetic construct
GGNYGDYFDYFDY

SEQ ID NO: 35 - protein, 6 aa, synthetic construct
QSYEGF

SEQ ID NO: 36 - protein, 13 aa, synthetic construct
TGRNGNIASNYVQ

SEQ ID NO: 37 - protein, 7 aa, synthetic construct
EDTQRPS

SEQ ID NO: 38 - protein, 9 aa, synthetic construct
QSSDSNRVL

SEQ ID NO: 39 - protein, 11 aa, synthetic construct
DFWVITSGNDY

SEQ ID NO: 40 - protein, 10 aa, synthetic construct
QSFDSTNLVV

SEQ ID NO: 41 - protein, 13 aa, synthetic construct
AGSSGSIASNYVQ

SEQ ID NO: 42 - protein, 10 aa, synthetic construct
QSYSYNNQVV

SEQ ID NO: 43 - DNA, 1362 bp, synthetic construct
  source 1..1362: mol_type = other DNA
gaggtgcagctgttggagtctgggggaggcttggtacagcctggggggtccctgagactctcctgtgcagcctctggattcacctttagcagctatgccatgagctgggtccgccaggctccagggaaggggctggagtgggtctcagctattagtggtagtggtggtagcacatactacgcagactccgtgaagggccggttcaccatctccagagacaattccaagaacacgctgtatctgcaaatgaacagcctgagagccgaggacacggccgtatattactgtgcgaaagatggtagcagtggctggtacgtaccacactggttcgacccctggggccagggaaccctggtcaccgtctcctcagcctccaccaagggcccatcggtcttccccctggcaccctcctccaagagcacctctgggggcacagcggccctgggctgcctggtcaaggactacttccccgaaccggtgacggtgtcgtggaactcaggcgccctgaccagcggcgtgcacaccttcccggctgtcctacagtcctcaggactctactccctcagcagcgtggtgaccgtgccctccagcagcttgggcacccagacctacatctgcaacgtgaatcacaagcccagcaacaccaaggtggacaagagagttgagcccaaatcttgtgacaaaactcacacatgcccaccgtgcccagcacctgaactcctggggggaccgtcagtcttcctcttccccccaaaacccaaggacaccctcatgatctcccggacccctgaggtcacatgcgtggtggtggacgtgagccacgaagaccctgaggtcaagttcaactggtacgtggacggcgtggaggtgcataatgccaagacaaagccgcgggaggagcagtacaacagcacgtaccgtgtggtcagcgtcctcaccgtcctgcaccaggactggctgaatggcaaggagtacaagtgcaaggtctccaacaaagccctcccagcccccatcgagaaaaccatctccaaagccaaagggcagccccgagaaccacaggtgtacaccctgcccccatcccgggaggagatgaccaagaaccaggtcagcctgacctgcctggtcaaaggcttctatcccagcgacatcgccgtggagtgggagagcaatgggcagccggagaacaactacaagaccacgcctcccgtgctggactccgacggctccttcttcctctatagcaagctcaccgtggacaagagcaggtggcagcaggggaacgtcttctcatgctccgtgatgcatgaggctctgcacaaccactacacgcagaagagcctctccctgtctccgggtaaatag

SEQ ID NO: 44 - protein, 453 aa, synthetic construct
EVQLLESGGGLVQPGGSLRLSCAASGFTFSSYAMSWVRQAPGKGLEWVSAISGSGGSTYYADSVKGRFTISRDNSKNTLYLQMNSLRAEDTAVYYCAKDGSSGWYVPHWFDPWGQGTLVTVSSASTKGPSVFPLAPSSKSTSGGTAALGCLVKDYFPEPVTVSWNSGALTSGVHTFPAVLQSSGLYSLSSVVTVPSSSLGTQTYICNVNHKPSNTKVDKRVEPKSCDKTHTCPPCPAPELLGGPSVFLFPPKPKDTLMISRTPEVTCVVVDVSHEDPEVKFNWYVDGVEVHNAKTKPREEQYNSTYRVVSVLTVLHQDWLNGKEYKCKVSNKALPAPIEKTISKAKGQPREPQVYTLPPSREEMTKNQVSLTCLVKGFYPSDIAVEWESNGQPENNYKTTPPVLDSDGSFFLYSKLTVDKSRWQQGNVFSCSVMHEALHNHYTQKSLSLSPGK

SEQ ID NO: 45 - DNA, 654 bp, synthetic construct
  source 1..654: mol_type = other DNA
aattttatgctgactcagccccactctgtgtcggagtctccggggaagacggtaaccatctcctgcactcgcagcagtggcagcattgccagcaactatgtgcagtggtaccaacagcgcccgggcagttcccccaccactgtcatctatgaggataaccagagaccctctggggtccctgatcggttctctggctccatcgacagctcctccaattctgcctccctcaccatctctgggctgaagactgaggacgaggctgactactactgtcagtcttatgatggcagcaatcgttggatgttcggcggagggaccaagctgaccgtcctaggtcagcccaaggctgccccctcggtcactctgttcccgccctcctctgaggagcttcaagccaacaaggccacactggtgtgtctcataagtgacttctacccgggagccgtgacagtggcctggaaggcagatagcagccccgtcaaggcgggagtggagaccaccacaccctccaaacaaagcaacaacaagtacgcggccagcagctacctgagcctgacgcctgagcagtggaagtcccacagaagctacagctgccaggtcacgcatgaagggagcaccgtggagaagacagtggcccctacagaatgttcatag

SEQ ID NO: 46 - protein, 217 aa, synthetic construct
NFMLTQPHSVSESPGKTVTISCTRSSGSIASNYVQWYQQRPGSSPTTVIYEDNQRPSGVPDRFSGSIDSSSNSASLTISGLKTEDEADYYCQSYDGSNRWMFGGGTKLTVLGQPKAAPSVTLFPPSSEELQANKATLVCLISDFYPGAVTVAWKADSSPVKAGVETTTPSKQSNNKYAASSYLSLTPEQWKSHRSYSCQVTHEGSTVEKTVAPTECS

SEQ ID NO: 47 - protein, 123 aa, synthetic construct
EVQLLESGGGLVQPGGSLRLSCAASGFTFSSYAMSWVRQAPGKGLEWVSAISGSGGSTYYADSVKGRFTISRDNSKNTLYLQMNSLRAEDTAVYYCAKDGSSGWYVPHWFDPWGQGTLVTVSS

SEQ ID NO: 48 - protein, 111 aa, synthetic construct
NFMLTQPHSVSESPGKTVTISCTRSSGSIASNYVQWYQQRPGSSPTTVIYEDNQRPSGVPDRFSGSIDSSSNSASLTISGLKTEDEADYYCQSYDGSNRWMFGGGTKLTVL

SEQ ID NO: 49 - DNA, 369 bp, synthetic construct
  source 1..369: mol_type = other DNA
gaggtgcagctgttggagtctgggggaggcttggtacagcctggggggtccctgagactctcctgtgcagcctctggattcacctttagcagctatgccatgagctgggtccgccaggctccagggaaggggctggagtgggtctcagctattagtggtagtggtggtagcacatactacgcagactccgtgaagggccggttcaccatctccagagacaattccaagaacacgctgtatctgcaaatgaacagcctgagagccgaggacacggccgtatattactgtgcgaaagatggtagcagtggctggtacgtaccacactggttcgacccctggggccggggcaccctggtcaccgtctcgagt

SEQ ID NO: 50 - protein, 123 aa, synthetic construct
EVQLLESGGGLVQPGGSLRLSCAASGFTFSSYAMSWVRQAPGKGLEWVSAISGSGGSTYYADSVKGRFTISRDNSKNTLYLQMNSLRAEDTAVYYCAKDGSSGWYVPHWFDPWGRGTLVTVSS

SEQ ID NO: 51 - DNA, 336 bp, synthetic construct
  source 1..336: mol_type = other DNA
aattttatgctgactcagccccactctgtgtcggagtctccggggaagacggtaaccatctcctgcactcgcagcagtggcagcattgtcagcaactatgtgcagtggtaccaacagcgcccgggcagtgcccccaccactgtcatctatgaggataaccggagaccctctggggtccctgatcggttctctggctccatcgacagctcctccaatactgcctccctcaccatctctgggctggaggctgaggacgaggctgactactactgtcagtcttatgatggcagcaatcgttggatgttcggcggagggaccaagctgaccgtcctaggt

SEQ ID NO: 52 - protein, 112 aa, synthetic construct
NFMLTQPHSVSESPGKTVTISCTRSSGSIVSNYVQWYQQRPGSAPTTVIYEDNRRPSGVPDRFSGSIDSSSNTASLTISGLEAEDEADYYCQSYDGSNRWMFGGGTKLTVLG

SEQ ID NO: 53 - DNA, 369 bp, synthetic construct
  source 1..369: mol_type = other DNA
gaggtgcagctgttggagtctgggggaggcttggtacagcctggggggtccctgagactctcctgtgcagcctctggattcacctttagcagctatgccatgagctgggtccgccaggctccagggaaggggctggagtgggtctcagctattagtggtagtggtggtagcacatactacgcagactccgtgaagggccggttcaccatctccagagacaattccaagaacacgctgtatctgcaaatgaacagcctgagagccgaggacacggccgtatattactgtgcgaaagatcatagcagtggctggtacgtaatctccggtatggacgtctggggccgagggacaatggtcaccgtctcgagt

SEQ ID NO: 54 - protein, 123 aa, synthetic construct
EVQLLESGGGLVQPGGSLRLSCAASGFTFSSYAMSWVRQAPGKGLEWVSAISGSGGSTYYADSVKGRFTISRDNSKNTLYLQMNSLRAEDTAVYYCAKDHSSGWYVISGMDVWGRGTMVTVSS

SEQ ID NO: 55 - DNA, 333 bp, synthetic construct
  source 1..333: mol_type = other DNA
aattttatgctgactcagccccactctgtgtcggagtctccggggaagacggtaaccatctcctgcacccgcagcagtggcagcattgccagcaactatgtgcagtggtaccagcagcgcccgggcagttcccccaccactgtgatctctgaggataaccaaagaccctctggggtccctgatcggttctctggctccgtcgacagctcctccaactctgcctccctcaccatttctggactgaggactgaggacgaggctgactattactgtcagtctaatgattccgacaatgtggttttcggcggagggaccaagctgaccgtcctaggt

SEQ ID NO: 56 - protein, 111 aa, synthetic construct
NFMLTQPHSVSESPGKTVTISCTRSSGSIASNYVQWYQQRPGSSPTTVISEDNQRPSGVPDRFSGSVDSSSNSASLTISGLRTEDEADYYCQSNDSDNVVFGGGTKLTVLG

SEQ ID NO: 57 - DNA, 366 bp, synthetic construct
  source 1..366: mol_type = other DNA
gaggtgcagctgttggagtctgggggaggcttggtacagcctggggggtccctgagactctcctgtgcagcctctggattcacctttagcagctatgccatgagctgggtccgccaggctccagggaaggggctggagtgggtctcagctattagtggtagtggtggtagcacatactacgcagactccgtgaagggccggttcaccatctccagagacaatcccaagaacacgctgtatctgcaaatgaacagcctgagagccgaggacacggccgtgtattactgtgcgaaggacctaacagtgggtggtccctggtactactttgactactggggccaaggaaccctggtcaccgtctcgagt

SEQ ID NO: 58 - protein, 122 aa, synthetic construct
EVQLLESGGGLVQPGGSLRLSCAASGFTFSSYAMSWVRQAPGKGLEWVSAISGSGGSTYYADSVKGRFTISRDNPKNTLYLQMNSLRAEDTAVYYCAKDLTVGGPWYYFDYWGQGTLVTVSS

SEQ ID NO: 59 - DNA, 333 bp, synthetic construct
  source 1..333: mol_type = other DNA
aattttatgctgactcagccccactctgtgtcggagtctccggggaagacggtaaccatctcctgcacccgcagcagtggcagcattgtcagcaactatgtgcagtggtaccagcagcgcccgggcagtgcccccaccactgtgatctttgacgatgaccaaagaccctctggggtccctggtcggttctctggctccctcgacagctcctccaactctgcctccctcaccatctctgggctgcagactgaggacgaggctgactactactgtcagtcttatgatagcagcaatgtggtattcggcggggggaccaaggtcaccgtcctaggt

SEQ ID NO: 60 - protein, 111 aa, synthetic construct
NFMLTQPHSVSESPGKTVTISCTRSSGSIVSNYVQWYQQRPGSAPTTVIFDDDQRPSGVPGRFSGSLDSSSNSASLTISGLQTEDEADYYCQSYDSSNVVFGGGTKVTVLG

SEQ ID NO: 61 - DNA, 360 bp, synthetic construct
  source 1..360: mol_type = other DNA
gaggtgcagctgttggagtctgggggaggcttggtacagcctggggggtccctgagactctcctgtgcagcctctggattcacctttagcagctatgccatgagctgggtccgccaggctccagggaaggggctggagtgggtctcagctattagtggtagtggtggtagcacatactacgcagactccgtgaagggccggttcaccatctccagagacaattccaagaacacgctgtatctgcaaatgaacagcctgagagccgaggacacggccgtgtattactgtgcgaaagatggatggaacgcgctgggatggcttgaatcctggggccggggcaccctggtcaccgtctcgagt

SEQ ID NO: 62 - protein, 120 aa, synthetic construct
EVQLLESGGGLVQPGGSLRLSCAASGFTFSSYAMSWVRQAPGKGLEWVSAISGSGGSTYYADSVKGRFTISRDNSKNTLYLQMNSLRAEDTAVYYCAKDGWNALGWLESWGRGTLVTVSS

SEQ ID NO: 63 - DNA, 336 bp, synthetic construct
  source 1..336: mol_type = other DNA
aattttatgctgactcagccccactctgtgtcggagtctccggggaggacgataaccatctcctgcacccgcagtggtggcagcattggcagctactatgtgcagtggtaccagcagcgcccgggcactgcccccaccactgtgatctatgacgataaaaaaagaccctctggggtccctgatcggttctctggctccatcgacagctcctccaactctgcctccctcaccatctctggactgaagactgaggacgaggctgactactattgtcagtcttatgatagcaacaatcttgtggttttcggcggagggaccaaggtcaccgtcctaggt

SEQ ID NO: 64 - protein, 112 aa, synthetic construct
NFMLTQPHSVSESPGRTITISCTRSGGSIGSYYVQWYQQRPGTAPTTVIYDDKKRPSGVPDRFSGSIDSSSNSASLTISGLKTEDEADYYCQSYDSNNLVVFGGGTKVTVLG

SEQ ID NO: 65 - DNA, 369 bp, synthetic construct
  source 1..369: mol_type = other DNA
gaggtgcagctgttggagtctgggggaggcttggtacagcctggggggtccctgagactctcctgtgcagcctctggattcacctttagcagctatgccatgagctgggtccgccaggctccagggaaggggctggagtgggtctcagctattagtggtagtggtggtagcacatactacgcagactccgtgaagggccggttcaccatctccagagacaattccaagaacacgctgtatctgcaaatgaacagcctgagagccgaggacacggccgtatattactgtgcgaaagatggtagcagtggctggtacgtaccacactggttcgacccctggggcagggggacaatggtcaccgtctcgagt

SEQ ID NO: 66 - protein, 123 aa, synthetic construct
EVQLLESGGGLVQPGGSLRLSCAASGFTFSSYAMSWVRQAPGKGLEWVSAISGSGGSTYYADSVKGRFTISRDNSKNTLYLQMNSLRAEDTAVYYCAKDGSSGWYVPHWFDPWGRGTMVTVSS

SEQ ID NO: 67 - DNA, 336 bp, synthetic construct
  source 1..336: mol_type = other DNA
aattttatgctgactcagccccactctgtgtcggagtctccggggaagacggtaaccatctcctgcacccgcagcagtggcaccattgccagcaactatgtgcagtggtaccagcagcgcccgggcagttcccccaccactgtgatctatgaggataaccaaagaccctctggggtccctgatcggttctctggctccatcgacagctcctccaactctgcctccctcaccatctctggactgaagactgaggacgaggctgactactactgtcagtcttatgataacagcaatcattgggtgttcggcggagggaccaaggtcaccgtcctaggt

SEQ ID NO: 68 - protein, 112 aa, synthetic construct
NFMLTQPHSVSESPGKTVTISCTRSSGTIASNYVQWYQQRPGSSPTTVIYEDNQRPSGVPDRFSGSIDSSSNSASLTISGLKTEDEADYYCQSYDNSNHWVFGGGTKVTVLG

SEQ ID NO: 69 - DNA, 360 bp, synthetic construct
  source 1..360: mol_type = other DNA
gaggtgcagctgttggagtctgggggaggcttggtacagccaggggggtccctgaaactctcctgtgcagcctctggattcacctttagcagcaatgccatgagttgggtccgccaggctccagggaaggggctggagtgggtctcaactcttactggtagtggtggtaccgcatactacgcagactccgtggagggccggttcagcatctccagagacaattccaagaacacactgtatctgcaaatgaacagcctgagagccgaggacacggccgtatattactgtgcgaagggcacggaactcgtgggaggaggacttgacaactggggccaaggcaccctggtcaccgtctcgagt

SEQ ID NO: 70 - protein, 120 aa, synthetic construct
EVQLLESGGGLVQPGGSLKLSCAASGFTFSSNAMSWVRQAPGKGLEWVSTLTGSGGTAYYADSVEGRFSISRDNSKNTLYLQMNSLRAEDTAVYYCAKGTELVGGGLDNWGQGTLVTVSS

SEQ ID NO: 71 - DNA, 339 bp, synthetic construct
  source 1..339: mol_type = other DNA
aattttatgctgactcagccccactctctgtcggagtctccggggaagacggtgacgatctcctgcaccggcagcggaggcagcattgccaccaactatgtgcagtggtatcagcagcgcccgggcagtgcccccaccactgtgatccatgaggataaccaaagaccctctggggtccctgatcggttctctggctccatcgacggctcctccaactctgcctccctcaccatctctggactgcagcctgaggacgaggctgattactactgtcagtcttatgatagtgacaatcatcatgtggtattcggcggagggaccaagctgaccgtcctaggt

SEQ ID NO: 72 - protein, 113 aa, synthetic construct
NFMLTQPHSLSESPGKTVTISCTGSGGSIATNYVQWYQQRPGSAPTTVIHEDNQRPSGVPDRFSGSIDGSSNSASLTISGLQPEDEADYYCQSYDSDNHHVVFGGGTKLTVLG

SEQ ID NO: 73 - DNA, 360 bp, synthetic construct
  source 1..360: mol_type = other DNA
gaggtgcagctgttggagtctgggggaggcttggtacagcctggggggtccctgagactctcctgtgcagcctctggattcacctttagcagctatgccatgagctgggtccgccaggctccagggaaggggctggagtgggtctcagctattagtggtagtggtggtagcacatactacgcagactccgtgaagggccggttcaccatctccagagacaattccaagaacacgctgtatctgcaaatgaacagcctgagagccgaggacacggccgtgtattactgtgcgaaagatggatggaacgcgctgggatggcttgaatcctggggcaaggggacaatggtcaccgtctcgagt

SEQ ID NO: 74 - protein, 120 aa, synthetic construct
EVQLLESGGGLVQPGGSLRLSCAASGFTFSSYAMSWVRQAPGKGLEWVSAISGSGGSTYYADSVKGRFTISRDNSKNTLYLQMNSLRAEDTAVYYCAKDGWNALGWLESWGKGTMVTVSS

SEQ ID NO: 75 - DNA, 339 bp, synthetic construct
  source 1..339: mol_type = other DNA
aattttatgctgactcagccccactctgtgtcggagtctccggggaagacggtaaccatctcctgcaccggcagcagtggcagcattgccagcaactatgtgcagtggtaccagcagcgcccgggcagtgcccccaccactgtgatctatgaggataaccaaagaccctctggggtccctgatcggttctctggctccatcgacagctcctccaactctgcctccctcaccatctctggactgaagactgaggacgaggctgactactactgtcagtcttatgatagcagcaatcaagaggtggtattcggcggagggaccaagctgaccgtcctaggt

SEQ ID NO: 76 - protein, 113 aa, synthetic construct
NFMLTQPHSVSESPGKTVTISCTGSSGSIASNYVQWYQQRPGSAPTTVIYEDNQRPSGVPDRFSGSIDSSSNSASLTISGLKTEDEADYYCQSYDSSNQEVVFGGGTKLTVLG

SEQ ID NO: 77 - DNA, 369 bp, synthetic construct
  source 1..369: mol_type = other DNA
gaggtgcagctgttggagtctgggggaggcttggtacagcctggggggtccctgagactctcctgtgcagcctctggattcacctttagcagctatgccatgagctgggtccgccaggctccagggaaggggctggagtgggtctcagctattagtggtagtggtggtagcacatactacgcagactccgtgaagggccggttcaccatctccagagacaattccaagaacacgctgtatctgcaaatgaacagcctgagagccgaggacacggccgtatattactgtgcgaaagatggtagcagtggctggtacgtaccacactggttcgacccctggggccagggaaccctggtcaccgtctcgagt

SEQ ID NO: 78 - protein, 123 aa, synthetic construct; identical to SEQ ID NO: 47

SEQ ID NO: 79 - DNA, 336 bp, synthetic construct
  source 1..336: mol_type = other DNA
aattttatgctgactcagccccactctgtgtcggagtctccggggaagacggttaccatctcctgcacccgcagcagtggcagcattgtcagcaactatgtacagtggtaccagcagcgcccgggcagttcccccaccactgtgatctatgaggataaccaaagaccctctggggtccctgatcggttctctggctccatcgacagctcctccaactctgcctccctcaccatctctggactgaagactgaggacgaggctgactactactgtcagtcttatgatagcaacaatttttgggtgttcggcggagggaccaagctgaccgtcctaggt

SEQ ID NO: 80 - protein, 112 aa, synthetic construct
NFMLTQPHSVSESPGKTVTISCTRSSGSIVSNYVQWYQQRPGSSPTTVIYEDNQRPSGVPDRFSGSIDSSSNSASLTISGLKTEDEADYYCQSYDSNNFWVFGGGTKLTVLG

SEQ ID NO: 81 - DNA, 360 bp, synthetic construct
  source 1..360: mol_type = other DNA
gaggtgcagctgttggagtctgggggaggcttggtacagcctggggggtccctgagactctcctgtgcagcctctggattcacctttagcagctatgccatgagctgggtccgccaggctccagggaaggggctggagtgggtctcagctattagtggtagtggtggtagcacatactacgcagactccgtgaagggccggttcaccatctccagagacaattccaagaacacgctgtatctgcaaatgaacagcctgagagccgaggacacggccgtgtattactgtgtgaaaaggtcctttgatagtggtgggtcctttgagtactggggccaggggacaatggtcaccgtctcgagt

SEQ ID NO: 82 - protein, 120 aa, synthetic construct
EVQLLESGGGLVQPGGSLRLSCAASGFTFSSYAMSWVRQAPGKGLEWVSAISGSGGSTYYADSVKGRFTISRDNSKNTLYLQMNSLRAEDTAVYYCVKRSFDSGGSFEYWGQGTMVTVSS

SEQ ID NO: 83 - DNA, 336 bp, synthetic construct
  source 1..336: mol_type = other DNA
aattttatgctgactcagccccactctgtgtcggagtctccggggaagacggtcaccatctcctgcacccgcagcagtggctacattgccagctcctatgtgcagtggtaccagcagcgcccgggcagttcccccaccactgtaatctttgaggatgaccggagaccctctggggtccctgatcggttctctggctccatcgacggctcctccaactctgcctccctcaccatctctggactgaggactgaggacgaggctgactactactgtcagtcttatgatgacaccactccctgggtgttcggcggagggaccaagctgaccgtcctaggt

SEQ ID NO: 84 - protein, 112 aa, synthetic construct
NFMLTQPHSVSESPGKTVTISCTRSSGYIASSYVQWYQQRPGSSPTTVIFEDDRRPSGVPDRFSGSIDGSSNSASLTISGLRTEDEADYYCQSYDDTTPWVFGGGTKLTVLG

SEQ ID NO: 85 - DNA, 360 bp, synthetic construct
  source 1..360: mol_type = other DNA
gaggtgcagctgttggagtctgggggaggcttggtacagcctggggggtccctgagactctcctgtgcagcctctggattcacctttagcagctatgccatgagctgggtccgccaggctccagggaaggggctggagtgggtctcagctattagtggtagtggtggtagcacatactacgcagactccgtgaagggccggttcaccatctccagagacaattccaagaacacgctgtatctgcaaatgaacagcctgagagccgaggacacggccgtgtattactgtgcgagagtcggcagctggtacctggaagattttgatatctggggccgggggacaatggtcaccgtctcgagt

SEQ ID NO: 86 - protein, 120 aa, synthetic construct
EVQLLESGGGLVQPGGSLRLSCAASGFTFSSYAMSWVRQAPGKGLEWVSAISGSGGSTYYADSVKGRFTISRDNSKNTLYLQMNSLRAEDTAVYYCARVGSWYLEDFDIWGRGTMVTVSS

SEQ ID NO: 87 - DNA, 342 bp, synthetic construct
  source 1..342: mol_type = other DNA
aattttatgctgactcagccccactctgtgtcggagtctccggggaagacggttaccatctcctgcacccgcagcagtggcagcattgccagcaactatgttcactggtatcagcagcgcccgggcagttcacccaccactgtgatctatgaggataaccgaagaccctctggggtccctgctcggttctctggctccatcgacagctcctccaactctgcctccctcaccatctctggactggagactgacgacgaggctgactactactgtcagtcttctgataccacctatcatggaggtgtggtattcggcggagggaccaagctgaccgtcctaggt

SEQ ID NO: 88 - protein, 114 aa, synthetic construct
NFMLTQPHSVSESPGKTVTISCTRSSGSIASNYVHWYQQRPGSSPTTVIYEDNRRPSGVPARFSGSIDSSSNSASLTISGLETDDEADYYCQSSDTTYHGGVVFGGGTKLTVLG

SEQ ID NO: 89 - DNA, 366 bp, synthetic construct
  source 1..366: mol_type = other DNA
gaggtgcagctgttggagtctgggggaggcttggtacagcctggggggtccctgagactctcctgtgcagcctctggattcacctttagcagctatgccatgagctgggtccgccaggctccagggaaggggctggagtgggtctcagctattagtggtagtggtggtagcacatactacgcagactccgtgaagggccggttcaccatctccagagacaattccaagaacacgctgtatctgcaaatgaacagcctgagagccgaggacacggccgtgtattactgtgcgaaaggcggtaactacggtgattacttcgactactttgactactggggcagagggacaatggtcaccgtctcgagt

SEQ ID NO: 90 - protein, 122 aa, synthetic construct
EVQLLESGGGLVQPGGSLRLSCAASGFTFSSYAMSWVRQAPGKGLEWVSAISGSGGSTYYADSVKGRFTISRDNSKNTLYLQMNSLRAEDTAVYYCAKGGNYGDYFDYFDYWGRGTMVTVSS

SEQ ID NO: 91 - DNA, 321 bp, synthetic construct
  source 1..321: mol_type = other DNA
aattttatgctgactcagccccactctgtgtcggagtctccggggaagacggtaaccatctcctgcacccgcagcagtggcagcattgccagcaattatgtgcagtggtaccagcagcgcccgggcagtgcccccaccattgtgatctatgaagataaccaaagaccctctggggtccctcatcggttctctggctccatcgacagctcctccaactctgcctccctcaccatctctggactgaagactgaggacgaggctgactactactgtcagtcttatgaggggttcggcggagggaccaagctgaccgtcctaggt

SEQ ID NO: 92 - protein, 107 aa, synthetic construct
NFMLTQPHSVSESPGKTVTISCTRSSGSIASNYVQWYQQRPGSAPTIVIYEDNQRPSGVPHRFSGSIDSSSNSASLTISGLKTEDEADYYCQSYEGFGGGTKLTVLG

SEQ ID NO: 93 - DNA, 360 bp, synthetic construct
  source 1..360: mol_type = other DNA
gaggtgcagctgttggagtctgggggaggcttggtacagcctggggggtccctgagactctcctgtgcagcctctggattcacctttagcagctatgccatgagctgggtccgccaggctccagggaaggggctggagtgggtctcagctattagtggtagtggtggtagcacatactacgcagactccgtgaagggccggttcactatctccagagacaattccaagaacacgctgtatctgcaaatgaacagcctgagagccgaggacacggccgtgtattactgtgcgaaagatggatggaacgcgctgggatggcttgaatcctggggccaggggacaatggtcaccgtctcgagt

SEQ ID NO: 94 - protein, 120 aa, synthetic construct
EVQLLESGGGLVQPGGSLRLSCAASGFTFSSYAMSWVRQAPGKGLEWVSAISGSGGSTYYADSVKGRFTISRDNSKNTLYLQMNSLRAEDTAVYYCAKDGWNALGWLESWGQGTMVTVSS

SEQ ID NO: 95 - DNA, 333 bp, synthetic construct
  source 1..333: mol_type = other DNA
aattttatgctgactcagccccacgctgtgtcggagtctccggggaagacggtgaccatttcctgcaccggcagaaatggcaacattgccagcaactatgtgcagtggtaccagcagcgcccggacagtgcccccacccttataatctttgaagatacccaaagaccctctggggtccctactcggctctcaggctccatcgacacctcctccaattctgcctccctcatcatctcttcattgaggactgaggacgaggctgattactactgtcaatcttctgattccaacagggtgctgttcggcggagggaccaaggtcaccgtcctaggt

SEQ ID NO: 96 - protein, 111 aa, synthetic construct
NFMLTQPHAVSESPGKTVTISCTGRNGNIASNYVQWYQQRPDSAPTLIIFEDTQRPSGVPTRLSGSIDTSSNSASLIISSLRTEDEADYYCQSSDSNRVLFGGGTKVTVLG

SEQ ID NO: 97 - DNA, 360 bp, synthetic construct
  source 1..360: mol_type = other DNA
gaggtgcagctgttggagtctgggggaggcttggtacagcctggggggtccctgagactctcctgtgcagcctctggattcacctttagcagctatgccatgagctgggtccgccaggctccagggaaggggctggagtgggtctcagctattagtggtagtggtggtagcacatactacgcagactccgtgaagggccggttcaccatctccagagacaattccaagaacacgctgtatctgcaaatgaacagcctgagagccgaggacacggccgtgtattactgtgcgaaagatttttgggttattacgagtgggaatgactactgggggcgggggaccacggtcaccgtctcgagt

SEQ ID NO: 98 - protein, 120 aa, synthetic construct
EVQLLESGGGLVQPGGSLRLSCAASGFTFSSYAMSWVRQAPGKGLEWVSAISGSGGSTYYADSVKGRFTISRDNSKNTLYLQMNSLRAEDTAVYYCAKDFWVITSGNDYWGRGTTVTVSS

SEQ ID NO: 99 - DNA, 336 bp, synthetic construct
  source 1..336: mol_type = other DNA
aattttatgctgactcagccccactctgtgtcggagtctccggggaagacggtgaccatctcctgcacccgcagcagtggcagcattgctagcaattatgtgcagtggtaccagcagcgcccgggcagttcccccaccactgtgatctttgaagataaccgaagaccctctggggtccctgatcggttttctggctccatcgacacctcctccaactctgcctccctcaccatctctggactgaagactgaggacgaggctgactactactgtcagtcttttgatagcaccaatcttgtggtgttcggcggagggaccaagctgaccgtcctaggt

SEQ ID NO: 100 - protein, 112 aa, synthetic construct
NFMLTQPHSVSESPGKTVTISCTRSSGSIASNYVQWYQQRPGSSPTTVIFEDNRRPSGVPDRFSGSIDTSSNSASLTISGLKTEDEADYYCQSFDSTNLVVFGGGTKLTVLG

SEQ ID NO: 101 - DNA, 360 bp, synthetic construct
  source 1..360: mol_type = other DNA
gaggtgcagctgttggagtctgggggaggcttggtacagcctggggggtccctgagactctcctgtgcagcctctggattcacctttagcagctatgccatgagctgggtccgccaggctccagggaaggggctggagtgggtctcagctattagtggtagtggtggtagcacatactacgcagactccgtgaagggccggttcaccatctccagagacaattccaagaacacgctgtatctgcaaatgaacagcctgagagccgaggacacggccgtgtattactgtgcgaaagatggatggaacgcgctgggatggcttgaatcctgggggaaggggaccacggtcaccgtctcgagt

SEQ ID NO: 102 - protein, 120 aa, synthetic construct
EVQLLESGGGLVQPGGSLRLSCAASGFTFSSYAMSWVRQAPGKGLEWVSAISGSGGSTYYADSVKGRFTISRDNSKNTLYLQMNSLRAEDTAVYYCAKDGWNALGWLESWGKGTTVTVSS

SEQ ID NO: 103 - DNA, 336 bp, synthetic construct
  source 1..336: mol_type = other DNA
aattttatgctgactcagccccactctgtgtcggagtctccggggaagacggtaaccatctcctgcgccggcagcagtggcagcattgccagcaactatgtgcagtggtaccagcagcgcccgggcagtgcccccaccgctgtgatctatgaggataaccaaagaccctctggggtccctgatcgattctctggctccatcgacagctcctccaactctgcctccctcaccatctctggactgaagactgaggacgaggctgactactactgtcaatcttactcttacaacaatcaggtcgtgttcggcggagggaccaaggtcaccgtcctaggt

SEQ ID NO: 104 - protein, 112 aa, synthetic construct
NFMLTQPHSVSESPGKTVTISCAGSSGSIASNYVQWYQQRPGSAPTAVIYEDNQRPSGVPDRFSGSIDSSSNSASLTISGLKTEDEADYYCQSYSYNNQVVFGGGTKVTVLG

SEQ ID NO: 105 - protein, 13 aa, synthetic construct
TRSSGYIASSYVQ